European Patent Application EP 4 553 084 A2, published May 14, 2025. Title: Use of IFN-Lambda mRNA for treating viral infections. Applicant: Ethris GmbH. Application EP. The sequence listing filed with the application follows.

SEQUENCE LISTING (42 sequences)

SEQ ID NO: 1 - RNA, 603 nt, Homo sapiens
  misc_feature 1..603: note = IFN Lambda 1
  source 1..603: mol_type = other RNA
  CDS 1..603: note = /transl_table=1
atggctgctgcttggacagtggtgctggtcacactggtgctgggacttgctgtggctggacctgtgcctaccagcaagcctaccacaacaggcaagggctgccacatcggcagattcaagagcctgtctcctcaagagctggcctccttcaagaaagccagggacgccctggaagagagcctgaagctgaagaactggtcctgcagcagccctgtgttccccggcaattgggatctgagactgctgcaagtgcgcgagaggcctgttgctctggaagctgaactggccctgacactgaaggtgctggaagccgctgctggacccgcactggaagatgttctggatcagcctctgcacaccctgcaccacattctgagtcagctgcaggcctgtatccagcctcagcctacagctggccctagacctagaggcagactgcaccactggctgcacagactgcaagaggcccctaagaaagagagcgccggctgtctggaagccagcgtgaccttcaacctgttcagactgctgacccgggacctgaaatacgtggccgatggcaatctgtgcctgcggacatctacacaccccgagagcacatga

SEQ ID NO: 2 - protein, 200 aa, Homo sapiens
  REGION 1..200: note = [CDS]:1..603 from SEQ ID NO 1
MAAAWTVVLVTLVLGLAVAGPVPTSKPTTTGKGCHIGRFKSLSPQELASFKKARDALEESLKLKNWSCSSPVFPGNWDLRLLQVRERPVALEAELALTLKVLEAAAGPALEDVLDQPLHTLHHILSQLQACIQPQPTAGPRPRGRLHHWLHRLQEAPKKESAGCLEASVTFNLFRLLTRDLKYVADGNLCLRTSTHPEST

SEQ ID NO: 3 - RNA, 603 nt, Homo sapiens
  misc_feature 1..603: note = IFN Lambda 2
  source 1..603: mol_type = other RNA
  CDS 1..603: note = /transl_table=1
atgaagctggacatgaccggcgattgcacccctgtgctggttctgatggctgccgtgctgacagtgacaggtgctgtgcctgtggctagactgcatggcgcactgcctgatgccagaggctgtcacattgcccagttcaagagcctgtctcctcaagagctgcaggccttcaagagagccaaggacgccctggaagagagcctgctgctgaaggattgccggtgccacagcagactgttccccagaacctgggacctgagacagctgcaagtgcgcgaaagacccatggctctggaagccgaactggccctgacactgaaagtgctggaagccaccgccgacaccgatcctgctctggtggatgttctggaccagcctctgcacaccctgcaccacatcctgagccagttcagggcctgtatccagcctcagcctacagctggccctagaaccagaggcagactgcaccactggctgtacagactgcaagaggcccctaagaaagagagccccggctgtctggaagctagcgtgaccttcaacctgttccggctgctgaccagggacctgaattgtgtggctagcggcgacctgtgcgtgtga

SEQ ID NO: 4 - protein, 200 aa, Homo sapiens
  REGION 1..200: note = [CDS]:1..603 from SEQ ID NO 3
MKLDMTGDCTPVLVLMAAVLTVTGAVPVARLHGALPDARGCHIAQFKSLSPQELQAFKRAKDALEESLLLKDCRCHSRLFPRTWDLRQLQVRERPMALEAELALTLKVLEATADTDPALVDVLDQPLHTLHHILSQFRACIQPQPTAGPRTRGRLHHWLYRLQEAPKKESPGCLEASVTFNLFRLLTRDLNCVASGDLCV

SEQ ID NO: 5 - RNA, 591 nt, Homo sapiens
  misc_feature 1..591: note = IFN Lambda 3
  source 1..591: mol_type = other RNA
  CDS 1..591: note = /transl_table=1
atgacaggcgattgcatgcctgtgctggtgctgatggctgccgtgctgacagttacaggtgctgtgcctgtggccagactgagaggtgcactgcctgatgccagaggctgtcacattgcccagttcaagagcctgtctcctcaagagctgcaggccttcaagagagccaaggacgccctggaagagagcctgctgctgaaggactgcaagtgcagaagccggctgttccccagaacctgggatctgagacagctgcaagtccgcgaaagacccgtggctctggaagctgaactggccctgacactgaaggtgctggaagccaccgccgataccgatcctgctctgggagatgtgctggaccagcctctgcacacactgcaccacatcctgagccagctgagggcctgtattcagccccaacctacagctggccctcggacaagaggcagactgcaccattggctgcaccggctgcaagaggcccctaagaaagagtctcctggctgcctggaagcctccgtgaccttcaacctgttcagactgctgacccgggacctgaattgtgtggcctctggcgatctgtgcgtgtga

SEQ ID NO: 6 - protein, 196 aa, Homo sapiens
  REGION 1..196: note = [CDS]:1..591 from SEQ ID NO 5
MTGDCMPVLVLMAAVLTVTGAVPVARLRGALPDARGCHIAQFKSLSPQELQAFKRAKDALEESLLLKDCKCRSRLFPRTWDLRQLQVRERPVALEAELALTLKVLEATADTDPALGDVLDQPLHTLHHILSQLRACIQPQPTAGPRTRGRLHHWLHRLQEAPKKESPGCLEASVTFNLFRLLTRDLNCVASGDLCV

SEQ ID NO: 7 - DNA, 13 bp, synthetic construct
  misc_feature 1..13: note = primer
  source 1..13: mol_type = other DNA
gggagacgccacc

SEQ ID NO: 8 - DNA, 17 bp, synthetic construct
  misc_feature 1..17: note = primer
  source 1..17: mol_type = other DNA
taatacgactcactata

SEQ ID NO: 9 - DNA, 30 bp, synthetic construct
  misc_feature 1..30: note = primer
  source 1..30: mol_type = other DNA
taatacgactcactatagggagacgccacc

SEQ ID NO: 10 - DNA, 637 bp, Homo sapiens
  misc_feature 1..637: note = DNA construct IFN Lambda 1
  source 1..637: mol_type = other DNA
taatacgactcactatagggagacgccaccatggctgctgcttggacagtggtgctggtcacactggtgctgggacttgctgtggctggacctgtgcctaccagcaagcctaccacaacaggcaagggctgccacatcggcagattcaagagcctgtctcctcaagagctggcctccttcaagaaagccagggacgccctggaagagagcctgaagctgaagaactggtcctgcagcagccctgtgttccccggcaattgggatctgagactgctgcaagtgcgcgagaggcctgttgctctggaagctgaactggccctgacactgaaggtgctggaagccgctgctggacccgcactggaagatgttctggatcagcctctgcacaccctgcaccacattctgagtcagctgcaggcctgtatccagcctcagcctacagctggccctagacctagaggcagactgcaccactggctgcacagactgcaagaggcccctaagaaagagagcgccggctgtctggaagccagcgtgaccttcaacctgttcagactgctgacccgggacctgaaatacgtggccgatggcaatctgtgcctgcggacatctacacaccccgagagcacatgattcg

SEQ ID NO: 11 - DNA, 637 bp, Homo sapiens
  misc_feature 1..637: note = DNA construct IFN Lambda 2
  source 1..637: mol_type = other DNA
taatacgactcactatagggagacgccaccatgaagctggacatgaccggcgattgcacccctgtgctggttctgatggctgccgtgctgacagtgacaggtgctgtgcctgtggctagactgcatggcgcactgcctgatgccagaggctgtcacattgcccagttcaagagcctgtctcctcaagagctgcaggccttcaagagagccaaggacgccctggaagagagcctgctgctgaaggattgccggtgccacagcagactgttccccagaacctgggacctgagacagctgcaagtgcgcgaaagacccatggctctggaagccgaactggccctgacactgaaagtgctggaagccaccgccgacaccgatcctgctctggtggatgttctggaccagcctctgcacaccctgcaccacatcctgagccagttcagggcctgtatccagcctcagcctacagctggccctagaaccagaggcagactgcaccactggctgtacagactgcaagaggcccctaagaaagagagccccggctgtctggaagctagcgtgaccttcaacctgttccggctgctgaccagggacctgaattgtgtggctagcggcgacctgtgcgtgtgattcg

SEQ ID NO: 12 - DNA, 625 bp, Homo sapiens
  misc_feature 1..625: note = DNA construct IFN Lambda 3
  source 1..625: mol_type = other DNA
taatacgactcactatagggagacgccaccatgacaggcgattgcatgcctgtgctggtgctgatggctgccgtgctgacagttacaggtgctgtgcctgtggccagactgagaggtgcactgcctgatgccagaggctgtcacattgcccagttcaagagcctgtctcctcaagagctgcaggccttcaagagagccaaggacgccctggaagagagcctgctgctgaaggactgcaagtgcagaagccggctgttccccagaacctgggatctgagacagctgcaagtccgcgaaagacccgtggctctggaagctgaactggccctgacactgaaggtgctggaagccaccgccgataccgatcctgctctgggagatgtgctggaccagcctctgcacacactgcaccacatcctgagccagctgagggcctgtattcagccccaacctacagctggccctcggacaagaggcagactgcaccattggctgcaccggctgcaagaggcccctaagaaagagtctcctggctgcctggaagcctccgtgaccttcaacctgttcagactgctgacccgggacctgaattgtgtggcctctggcgatctgtgcgtgtgattcg

SEQ ID NO: 13 - RNA, 620 nt, Homo sapiens
  misc_feature 1..620: note = mRNA construct for IFN Lambda 1
  source 1..620: mol_type = other RNA
gggagacgccaccatggctgctgcttggacagtggtgctggtcacactggtgctgggacttgctgtggctggacctgtgcctaccagcaagcctaccacaacaggcaagggctgccacatcggcagattcaagagcctgtctcctcaagagctggcctccttcaagaaagccagggacgccctggaagagagcctgaagctgaagaactggtcctgcagcagccctgtgttccccggcaattgggatctgagactgctgcaagtgcgcgagaggcctgttgctctggaagctgaactggccctgacactgaaggtgctggaagccgctgctggacccgcactggaagatgttctggatcagcctctgcacaccctgcaccacattctgagtcagctgcaggcctgtatccagcctcagcctacagctggccctagacctagaggcagactgcaccactggctgcacagactgcaagaggcccctaagaaagagagcgccggctgtctggaagccagcgtgaccttcaacctgttcagactgctgacccgggacctgaaatacgtggccgatggcaatctgtgcctgcggacatctacacaccccgagagcacatgattcg

SEQ ID NO: 14 - RNA, 620 nt, Homo sapiens
  misc_feature 1..620: note = mRNA construct for IFN Lambda 2
  source 1..620: mol_type = other RNA
gggagacgccaccatgaagctggacatgaccggcgattgcacccctgtgctggttctgatggctgccgtgctgacagtgacaggtgctgtgcctgtggctagactgcatggcgcactgcctgatgccagaggctgtcacattgcccagttcaagagcctgtctcctcaagagctgcaggccttcaagagagccaaggacgccctggaagagagcctgctgctgaaggattgccggtgccacagcagactgttccccagaacctgggacctgagacagctgcaagtgcgcgaaagacccatggctctggaagccgaactggccctgacactgaaagtgctggaagccaccgccgacaccgatcctgctctggtggatgttctggaccagcctctgcacaccctgcaccacatcctgagccagttcagggcctgtatccagcctcagcctacagctggccctagaaccagaggcagactgcaccactggctgtacagactgcaagaggcccctaagaaagagagccccggctgtctggaagctagcgtgaccttcaacctgttccggctgctgaccagggacctgaattgtgtggctagcggcgacctgtgcgtgtgattcg

SEQ ID NO: 15 - RNA, 597 nt, Homo sapiens
  misc_feature 1..597: note = mRNA construct for IFN Lambda 3
  source 1..597: mol_type = other RNA
gggagacgccaccatgacaggcgattgcatgcctgtgctggtgctgatggctgccgtgctgacagttacaggtgctgtgcctgtggccagactgagaggtgcactgcctgatgccagaggctgtcacattgcccagttcaagagcctgtctcctcaagagctgcaggccttcaagagagccaaggacgccctggaagagagcctgctgctgaaggactgcaagtgcagaagccggctgttccccagaacctgggatctgagacagctgcaagtccgcgaaagacccgtggctctggaagctgaactggccctgacactgaaggtgctggaagccaccgccgataccgatcctgctctgggagatgtgctggaccagcctctgcacacactgcaccacatcctgagccagctgagggcctgtattcagccccaacctacagctggccctcggacaagaggcagactgcaccattggctgcaccggctgcaagaggcccctaagaaagagtctcctggctgcctggaagcctccgtgaccttcaacctgttcagactgctgacccgggacctgaattgtgtggcctctggcgatctgtg

SEQ ID NO: 16 - RNA, 570 nt, Homo sapiens
  misc_feature 1..570: note = IFN alpha 16
  source 1..570: mol_type = other RNA
  CDS 1..570: note = /transl_table=1
atggccctgagcttctctctgctgatggctgtgctggtgctgagctacaagagcatctgcagcctgggctgcgacctgcctcagacacactctctgggaaacagacgggccctgattctgctggcccagatgggcagaatctcccacttcagctgcctgaaggacagatacgacttcggcttccctcaagaggtgttcgacggcaaccagttccagaaggcccaggccatctctgccttccacgagatgatccagcagaccttcaacctgttcagcaccaaggatagcagcgccgcctgggatgagacactgctggacaagttctacatcgagctgttccagcagctgaacgacctggaagcctgcgtgacacaagaagtgggcgtcgaagagatcgccctgatgaacgaggatagcatcctggccgtgcgcaagtacttccagcggatcaccctgtacctgatgggcaagaagtacagcccttgcgcctgggaagtcgtgcgggccgaaatcatgagaagcttcagctttagcaccaacctgcagaagggcctgagaagaaaggactga

SEQ ID NO: 17 - protein, 189 aa, Homo sapiens
  REGION 1..189: note = [CDS]:1..570 from SEQ ID NO 16
MALSFSLLMAVLVLSYKSICSLGCDLPQTHSLGNRRALILLAQMGRISHFSCLKDRYDFGFPQEVFDGNQFQKAQAISAFHEMIQQTFNLFSTKDSSAAWDETLLDKFYIELFQQLNDLEACVTQEVGVEEIALMNEDSILAVRKYFQRITLYLMGKKYSPCAWEVVRAEIMRSFSFSTNLQKGLRRKD

SEQ ID NO: 18 - RNA, 564 nt, Homo sapiens
  misc_feature 1..564: note = IFN beta
  source 1..564: mol_type = other RNA
  CDS 1..564: note = /transl_table=1
atgaccaacaagtgcctgctgcagattgccctgctgctgtgcttcagcacaacagccctgagcatgagctacaacctgctgggcttcctgcagcggagcagcaacttccagtgccagaaactgctgtggcagctgaacggccggctggaatactgcctgaaggaccggatgaacttcgacatccccgaggaaatcaagcagctgcagcagttccagaaagaggacgccgctctgaccatctacgagatgctgcagaacatcttcgccatcttccggcaggacagcagctccacaggctggaacgagacaatcgtggaaaatctgctggccaacgtgtaccaccagatcaaccacctgaaaaccgtgctggaagagaagctggaaaaagaggacttcacccggggcaagctgatgagcagcctgcacctgaagcggtactacggcagaatcctgcactacctgaaggccaaagagtacagccactgcgcctggaccatcgtgcgcgtggaaatcctgcggaacttctacttcatcaaccggctgaccggctacctgagaaactga

SEQ ID NO: 19 - protein, 187 aa, Homo sapiens
  REGION 1..187: note = [CDS]:1..564 from SEQ ID NO 18
MTNKCLLQIALLLCFSTTALSMSYNLLGFLQRSSNFQCQKLLWQLNGRLEYCLKDRMNFDIPEEIKQLQQFQKEDAALTIYEMLQNIFAIFRQDSSSTGWNETIVENLLANVYHQINHLKTVLEEKLEKEDFTRGKLMSSLHLKRYYGRILHYLKAKEYSHCAWTIVRVEILRNFYFINRLTGYLRN

SEQ ID NO: 20 - RNA, 501 nt, Homo sapiens
  misc_feature 1..501: note = IFN gamma
  source 1..501: mol_type = other RNA
  CDS 1..501: note = /transl_table=1
atgaagtacaccagctacatcctggccttccagctgtgcatcgtgctgggaagcctgggctgctactgccaggatccttacgtgaaagaggccgagaacctgaagaagtactttaacgccggccacagcgacgtggccgacaatggaacactgttcctgggcatcctgaagaactggaaagaggaaagcgaccggaagatcatgcagagccagatcgtgtccttctacttcaagctgttcaagaacttcaaggacgaccagagcatccagaaaagcgtggaaaccatcaaagaagatatgaacgtcaagttcttcaactccaacaagaagaagcgggacgacttcgagaagctgaccaactacagcgtgaccgacctgaacgtgcagagaaaggccatccacgagctgatccaagtgatggccgaactgtctcctgccgccaagaccggaaagcggaagagaagccagatgctgttcagaggcagacgggcctctcagtga

SEQ ID NO: 21 - protein, 166 aa, Homo sapiens
  REGION 1..166: note = [CDS]:1..501 from SEQ ID NO 20
MKYTSYILAFQLCIVLGSLGCYCQDPYVKEAENLKKYFNAGHSDVADNGTLFLGILKNWKEESDRKIMQSQIVSFYFKLFKNFKDDQSIQKSVETIKEDMNVKFFNSNKKKRDDFEKLTNYSVTDLNVQRKAIHELIQVMAELSPAAKTGKRKRSQMLFRGRRASQ

SEQ ID NO: 22 - DNA, 604 bp, Homo sapiens
  misc_feature 1..604: note = DNA construct IFN alpha 16
  source 1..604: mol_type = other DNA
taatacgactcactatagggagacgccaccatggccctgagcttctctctgctgatggctgtgctggtgctgagctacaagagcatctgcagcctgggctgcgacctgcctcagacacactctctgggaaacagacgggccctgattctgctggcccagatgggcagaatctcccacttcagctgcctgaaggacagatacgacttcggcttccctcaagaggtgttcgacggcaaccagttccagaaggcccaggccatctctgccttccacgagatgatccagcagaccttcaacctgttcagcaccaaggatagcagcgccgcctgggatgagacactgctggacaagttctacatcgagctgttccagcagctgaacgacctggaagcctgcgtgacacaagaagtgggcgtcgaagagatcgccctgatgaacgaggatagcatcctggccgtgcgcaagtacttccagcggatcaccctgtacctgatgggcaagaagtacagcccttgcgcctgggaagtcgtgcgggccgaaatcatgagaagcttcagctttagcaccaacctgcagaagggcctgagaagaaaggactgattcg

SEQ ID NO: 23 - DNA, 598 bp, Homo sapiens
  misc_feature 1..598: note = DNA construct IFN beta
  source 1..598: mol_type = other DNA
taatacgactcactatagggagacgccaccatgaccaacaagtgcctgctgcagattgccctgctgctgtgcttcagcacaacagccctgagcatgagctacaacctgctgggcttcctgcagcggagcagcaacttccagtgccagaaactgctgtggcagctgaacggccggctggaatactgcctgaaggaccggatgaacttcgacatccccgaggaaatcaagcagctgcagcagttccagaaagaggacgccgctctgaccatctacgagatgctgcagaacatcttcgccatcttccggcaggacagcagctccacaggctggaacgagacaatcgtggaaaatctgctggccaacgtgtaccaccagatcaaccacctgaaaaccgtgctggaagagaagctggaaaaagaggacttcacccggggcaagctgatgagcagcctgcacctgaagcggtactacggcagaatcctgcactacctgaaggccaaagagtacagccactgcgcctggaccatcgtgcgcgtggaaatcctgcggaacttctacttcatcaaccggctgaccggctacctgagaaactgattcg

SEQ ID NO: 24 - DNA, 535 bp, Homo sapiens
  misc_feature 1..535: note = DNA construct IFN gamma
  source 1..535: mol_type = other DNA
taatacgactcactatagggagacgccaccatgaagtacaccagctacatcctggccttccagctgtgcatcgtgctgggaagcctgggctgctactgccaggatccttacgtgaaagaggccgagaacctgaagaagtactttaacgccggccacagcgacgtggccgacaatggaacactgttcctgggcatcctgaagaactggaaagaggaaagcgaccggaagatcatgcagagccagatcgtgtccttctacttcaagctgttcaagaacttcaaggacgaccagagcatccagaaaagcgtggaaaccatcaaagaagatatgaacgtcaagttcttcaactccaacaagaagaagcgggacgacttcgagaagctgaccaactacagcgtgaccgacctgaacgtgcagagaaaggccatccacgagctgatccaagtgatggccgaactgtctcctgccgccaagaccggaaagcggaagagaagccagatgctgttcagaggcagacgggcctctcagtgattcg

SEQ ID NO: 25 - RNA, 587 nt, Homo sapiens
  misc_feature 1..587: note = mRNA construct for IFN alpha 16
  source 1..587: mol_type = other RNA
gggagacgccaccatggccctgagcttctctctgctgatggctgtgctggtgctgagctacaagagcatctgcagcctgggctgcgacctgcctcagacacactctctgggaaacagacgggccctgattctgctggcccagatgggcagaatctcccacttcagctgcctgaaggacagatacgacttcggcttccctcaagaggtgttcgacggcaaccagttccagaaggcccaggccatctctgccttccacgagatgatccagcagaccttcaacctgttcagcaccaaggatagcagcgccgcctgggatgagacactgctggacaagttctacatcgagctgttccagcagctgaacgacctggaagcctgcgtgacacaagaagtgggcgtcgaagagatcgccctgatgaacgaggatagcatcctggccgtgcgcaagtacttccagcggatcaccctgtacctgatgggcaagaagtacagcccttgcgcctgggaagtcgtgcgggccgaaatcatgagaagcttcagctttagcaccaacctgcagaagggcctgagaagaaaggactgattcg

SEQ ID NO: 26 - RNA, 581 nt, Homo sapiens
  misc_feature 1..581: note = mRNA construct for IFN beta
  source 1..581: mol_type = other RNA
gggagacgccaccatgaccaacaagtgcctgctgcagattgccctgctgctgtgcttcagcacaacagccctgagcatgagctacaacctgctgggcttcctgcagcggagcagcaacttccagtgccagaaactgctgtggcagctgaacggccggctggaatactgcctgaaggaccggatgaacttcgacatccccgaggaaatcaagcagctgcagcagttccagaaagaggacgccgctctgaccatctacgagatgctgcagaacatcttcgccatcttccggcaggacagcagctccacaggctggaacgagacaatcgtggaaaatctgctggccaacgtgtaccaccagatcaaccacctgaaaaccgtgctggaagagaagctggaaaaagaggacttcacccggggcaagctgatgagcagcctgcacctgaagcggtactacggcagaatcctgcactacctgaaggccaaagagtacagccactgcgcctggaccatcgtgcgcgtggaaatcctgcggaacttctacttcatcaaccggctgaccggctacctgagaaactgattcg

SEQ ID NO: 27 - RNA, 518 nt, Homo sapiens
  misc_feature 1..518: note = mRNA construct for IFN gamma
  source 1..518: mol_type = other RNA
gggagacgccaccatgaagtacaccagctacatcctggccttccagctgtgcatcgtgctgggaagcctgggctgctactgccaggatccttacgtgaaagaggccgagaacctgaagaagtactttaacgccggccacagcgacgtggccgacaatggaacactgttcctgggcatcctgaagaactggaaagaggaaagcgaccggaagatcatgcagagccagatcgtgtccttctacttcaagctgttcaagaacttcaaggacgaccagagcatccagaaaagcgtggaaaccatcaaagaagatatgaacgtcaagttcttcaactccaacaagaagaagcgggacgacttcgagaagctgaccaactacagcgtgaccgacctgaacgtgcagagaaaggccatccacgagctgatccaagtgatggccgaactgtctcctgccgccaagaccggaaagcggaagagaagccagatgctgttcagaggcagacgggcctctcagtgattcg

SEQ ID NO: 28 - DNA, 24 bp, synthetic construct
  misc_feature 1..24: note = M+24 F primer
  source 1..24: mol_type = other DNA
agatgagtcttctaaccgaggtcg

SEQ ID NO: 29 - DNA, 24 bp, synthetic construct
  misc_feature 1..24: note = Rev-mod primer
  source 1..24: mol_type = other DNA
tgcaaagacactttccagtctctg

SEQ ID NO: 30 - DNA, 20 bp, synthetic construct
  misc_feature 1..20: note = M+64 probe
  source 1..20: mol_type = other DNA
tcaggccccctcaaagccga

SEQ ID NO: 31 - DNA, 20 bp, synthetic construct
  misc_feature 1..20: note = Fer_GAPDH FWD primer
  source 1..20: mol_type = other DNA
caacggatttggccgtattg

SEQ ID NO: 32 - DNA, 23 bp, synthetic construct
  misc_feature 1..23: note = Fer_GAPDH REV primer
  source 1..23: mol_type = other DNA
ctggaacatgtagaccatgtagt

SEQ ID NO: 33 - DNA, 27 bp, synthetic construct
  misc_feature 1..27: note = Fer_GAPDH PRB probe
  source 1..27: mol_type = other DNA
agggtcattgatggcgacaatatccac

SEQ ID NO: 34 - DNA, 20 bp, synthetic construct
  misc_feature 1..20: note = SARS-CoV-2 N gene qPCR primer 1
  source 1..20: mol_type = other DNA
aaattttggggaccaggaac

SEQ ID NO: 35 - DNA, 20 bp, synthetic construct
  misc_feature 1..20: note = SARS-CoV-2 N gene qPCR primer 2
  source 1..20: mol_type = other DNA
tggcacctgtgtaggtcaac

SEQ ID NO: 36 - DNA, 20 bp, synthetic construct
  misc_feature 1..20: note = SARS-CoV-2 N gene qPCR probe
  source 1..20: mol_type = other DNA
atgtcgcgcattggcatgga

SEQ ID NO: 37 - protein, 200 aa, synthetic construct; identical to SEQ ID NO: 2
  source 1..200: note = The sequence is a translation of SEQ ID NO: 3.

SEQ ID NO: 38 - protein, 200 aa, synthetic construct; identical to SEQ ID NO: 4
  source 1..200: note = The sequence is a translation of SEQ ID NO: 3.

SEQ ID NO: 39 - protein, 196 aa, synthetic construct; identical to SEQ ID NO: 6
  source 1..196: note = The sequence is a translation of SEQ ID NO: 5.

SEQ ID NO: 40 - protein, 189 aa, synthetic construct; identical to SEQ ID NO: 17
  source 1..189: note = The the sequence is a translation of SEQ ID NO: 16.

SEQ ID NO: 41 - protein, 187 aa, synthetic construct; identical to SEQ ID NO: 19
  source 1..187: note = The sequence is a translation of SEQ ID NO: 18.

SEQ ID NO: 42 - protein, 166 aa, synthetic construct; identical to SEQ ID NO: 21
  source 1..166: note = The sequence is a translation of SEQ ID NO: 20.